European Patent Application EP 4 545 525 A1, published April 30, 2025. Title: Compounds and pharmaceutical compositions for treating autoimmune diseases. Applicant: 파렌키마바이오텍 주식회사. Application KR. The sequence listing filed with the application follows.

SEQUENCE LISTING (28 sequences)

SEQ ID NO: 1 - DNA, 23 bp, synthetic construct
  source 1..23: mol_type = other DNA
caccctcatcagtaatggtcaga

SEQ ID NO: 2 - DNA, 20 bp, synthetic construct
  source 1..20: mol_type = other DNA
aacgtgcttatcaggacctc

SEQ ID NO: 3 - DNA, 20 bp, synthetic construct
  source 1..20: mol_type = other DNA
tgatgacatcaagaaggtgg

SEQ ID NO: 4 - DNA, 20 bp, synthetic construct
  source 1..20: mol_type = other DNA
ttactccttggaggccatgt

SEQ ID NO: 5 - DNA, 22 bp, synthetic construct
  source 1..22: mol_type = other DNA
gatggctgaaaaagatggatgc

SEQ ID NO: 6 - DNA, 20 bp, synthetic construct
  source 1..20: mol_type = other DNA
tggttgggtcaggggtggtt

SEQ ID NO: 7 - DNA, 21 bp, synthetic construct
  source 1..21: mol_type = other DNA
ctcgtgctgtcggacccatat

SEQ ID NO: 8 - DNA, 22 bp, synthetic construct
  source 1..22: mol_type = other DNA
ttgaagacaaaccgcttttcca

SEQ ID NO: 9 - DNA, 22 bp, synthetic construct
  source 1..22: mol_type = other DNA
catgttctctgcgaaatcgtgg

SEQ ID NO: 10 - DNA, 22 bp, synthetic construct
  source 1..22: mol_type = other DNA
aacgcactaggtttgccgagta

SEQ ID NO: 11 - DNA, 21 bp, synthetic construct
  source 1..21: mol_type = other DNA
tttaactcccttggcgcaaaa

SEQ ID NO: 12 - DNA, 20 bp, synthetic construct
  source 1..20: mol_type = other DNA
ctttccctccgcattgacac

SEQ ID NO: 13 - DNA, 20 bp, synthetic construct
  source 1..20: mol_type = other DNA
ccacaccgtcagccgatttg

SEQ ID NO: 14 - DNA, 21 bp, synthetic construct
  source 1..21: mol_type = other DNA
cacccattcccttcacagagc

SEQ ID NO: 15 - DNA, 22 bp, synthetic construct
  source 1..22: mol_type = other DNA
aaatcaccatgccctctacaag

SEQ ID NO: 16 - DNA, 22 bp, synthetic construct
  source 1..22: mol_type = other DNA
cccacttttatcaccatcgcaa

SEQ ID NO: 17 - DNA, 23 bp, synthetic construct
  source 1..23: mol_type = other DNA
atactctaggaaggaaggacacc

SEQ ID NO: 18 - DNA, 23 bp, synthetic construct
  source 1..23: mol_type = other DNA
tccatgatgtcatttatgagggc

SEQ ID NO: 19 - DNA, 21 bp, synthetic construct
  source 1..21: mol_type = other DNA
caaggcagtggagcaggtgaa

SEQ ID NO: 20 - DNA, 23 bp, synthetic construct
  source 1..23: mol_type = other DNA
cggagagaggtacaaacgaggtt

SEQ ID NO: 21 - DNA, 19 bp, synthetic construct
  source 1..19: mol_type = other DNA
cccatccccaggagtcttg

SEQ ID NO: 22 - DNA, 21 bp, synthetic construct
  source 1..21: mol_type = other DNA
accatgactaggggcactgta

SEQ ID NO: 23 - DNA, 23 bp, synthetic construct
  source 1..23: mol_type = other DNA
actccctgaagaatataccctcc

SEQ ID NO: 24 - DNA, 22 bp, synthetic construct
  source 1..22: mol_type = other DNA
cgctattgagcacagatacgag

SEQ ID NO: 25 - DNA, 20 bp, synthetic construct
  source 1..20: mol_type = other DNA
atgcccacctcctcaaagac

SEQ ID NO: 26 - DNA, 23 bp, synthetic construct
  source 1..23: mol_type = other DNA
gtagtttccgttggaacagtgaa

SEQ ID NO: 27 - DNA, 20 bp, synthetic construct
  source 1..20: mol_type = other DNA
ttcaccaccatggagaaggc

SEQ ID NO: 28 - DNA, 20 bp, synthetic construct
  source 1..20: mol_type = other DNA
ggcatggactgtggtcatga